European Patent Application EP 4 545 083 A1, published April 30, 2025. Title: Composition for inhibiting peritoneal deterioration, composition kit for inhibiting peritoneal deterioration, peritoneal dialysis solution, and peritoneal dialysis solution kit. Applicant: 学校法人　愛知医科大学. Application JP. The sequence listing filed with the application follows.

SEQUENCE LISTING (12 sequences)

SEQ ID NO: 1 - DNA, 20 bp, synthetic construct
  misc_feature 1..20: note = Forwad primer for VEGF-A
  source 1..20: mol_type = other DNA
caggctgctgtaacgatgaa

SEQ ID NO: 2 - DNA, 20 bp, synthetic construct
  misc_feature 1..20: note = Reverse primer for VEGF-A
  source 1..20: mol_type = other DNA
gctttggtgaggtttgatcc

SEQ ID NO: 3 - DNA, 27 bp, synthetic construct
  misc_feature 1..27: note = Forward primer for VEGF-C
  source 1..27: mol_type = other DNA
cagacaagttcattcaattattagacg

SEQ ID NO: 4 - DNA, 21 bp, synthetic construct
  misc_feature 1..21: note = Reverse primer for VEGF-C
  source 1..21: mol_type = other DNA
catgtcttgttagctgcctga

SEQ ID NO: 5 - DNA, 18 bp, synthetic construct
  misc_feature 1..18: note = Fowrard primer for PECAM-1
  source 1..18: mol_type = other DNA
cggtgttcagcgagatcc

SEQ ID NO: 6 - DNA, 21 bp, synthetic construct
  misc_feature 1..21: note = Reverse primer for PECAM-1
  source 1..21: mol_type = other DNA
actcgacaggatggaaatcac

SEQ ID NO: 7 - DNA, 19 bp, synthetic construct
  misc_feature 1..19: note = Forward primer for LYVE-1
  source 1..19: mol_type = other DNA
gaagcagctgggtttggag

SEQ ID NO: 8 - DNA, 19 bp, synthetic construct
  misc_feature 1..19: note = Reverse primer for LYVE-1
  source 1..19: mol_type = other DNA
cgtagcaaacagccagcac

SEQ ID NO: 9 - DNA, 25 bp, synthetic construct
  misc_feature 1..25: note = Forward primer for IL-6
  source 1..25: mol_type = other DNA
gctaccaaactggatataatcagga

SEQ ID NO: 10 - DNA, 24 bp, synthetic construct
  misc_feature 1..24: note = Reverse primer for IL-6
  source 1..24: mol_type = other DNA
ccaggtagctatggtactccagaa

SEQ ID NO: 11 - DNA, 20 bp, synthetic construct
  misc_feature 1..20: note = Forward primer for GAPDH
  source 1..20: mol_type = other DNA
tgtgtccgtcgtggatctga

SEQ ID NO: 12 - DNA, 21 bp, synthetic construct
  misc_feature 1..21: note = Reverse primer for GAPDH
  source 1..21: mol_type = other DNA
ttgctgttgaagtcgcaggag